European Patent Specification EP 3 636 735 B1, published March 27, 2024. Title: PROTEASE ENZYME VARIANTS AND USES THEREOF. Applicant: AB Enzymes GmbH. The sequence listing filed with the application follows.

SEQUENCE LISTING (10 sequences)

SEQ ID NO: 1 - DNA, 1004 bp, Malbranchea cinnamomea
  mature protease nucleotide sequence
gcattggtgacgcagagtaatgcaccatcctggggccttggccgtatttccaaccgacaggctggtattcgtgattaccactacgatgactccgccggtgaaggcgtcatcgtctatgatgttgacaccggcattgacatcagccatccggatttcgagggccgtgctatatggggttccaaccatgtcgaccgcgttaaccaggatcagaatggccatgggacacacgttgctggtactattggtggaagggcgtacggagtcgccaagaaggccacaatagtggctgtcaaggttctcgacgcccaggggtcaggtactatcagcggtattattgctggtcttgactggagtgtcaatcatgctcgacagaatggagtcactagaagagcggctttgaacatgagccttggcggtgggcgcagtatctctttcaatcaggctgctgcaagtgctgtccaagccggattgttcgtcgcggttgctgccggaaatgaaggggtaagtgacttctttctggcccctcctatccgtacctgcagaagctaaccagattgctcttattttttttcttttttcaaaatatagcaaaatgcaggtaacacttccccagcctcagagccttctgtttgcacagtaggggcaacctcatcgaatgatgccgccacatcctggtccaactatggctcagttggtacgtagggctcggttttatttattacttcttccccacatgcgatcagaccggccgctgactatatttagttgacgtttacgctcccggagacgcaattgtctctacctggcccggtggcggttccaggtctctctcaggcacatcgatggcttctccacacgtcgccggcctgggtgcatacctcatcgctctggagggcattagcggaggcagtgtatgtgaccgtatcaaagagctggctcaacctgtcgtccagcctggtccaggcaccaccaaccgtcttatctacaacggcagtggccgctaa

SEQ ID NO: 2 - protein, 281 aa, Malbranchea cinnamomea
  mature protease amino acid sequence
ALVTQSNAPSWGLGRISNRQAGIRDYHYDDSAGEGVIVYDVDTGIDISHPDFEGRAIWGSNHVDRVNQDQNGHGTHVAGTIGGRAYGVAKKATIVAVKVLDAQGSGTISGIIAGLDWSVNHARQNGVTRRAALNMSLGGGRSISFNQAAASAVQAGLFVAVAAGNEGQNAGNTSPASEPSVCTVGATSSNDAATSWSNYGSVVDVYAPGDAIVSTWPGGGSRSLSGTSMASPHVAGLGAYLIALEGISGGSVCDRIKELAQPVVQPGPGTTNRLIYNGSGR

SEQ ID NO: 3 - DNA, 1004 bp, Malbranchea cinnamomea
  M59 mature nucleotide sequence
  misc_feature
  224: (309)..(309)
  225: r is t or c
gcattggtgacgcagagtaatgcaccatcctggggccttggccgtatttccaaccgacaggctggtattcgtgattaccactacgatgactccgccggtgaaggcgtcatcgtctatgatgttgacaccggcattgacatcagccatccggatttcgagggccgtgctatatggggttccaaccatgtcgaccgcgttaaccaggatcagaatggccatgggacacacgttgctggtactattggtggaagggcgtacggagtcgccaagaaggccacaatagtggctgtcaaggttctcgacgccgargggtcaggtactatcagcggtattattgctggtcttgactggagtgtcaatcatgctcgacagaatggagtcactagaagagcggctttgaacatgagccttggcggtgggcgcagtatctctttcaatcaggctgctgcaagtgctgtccaagccggattgttcgtcgcggttgctgccggaaatgaaggggtaagtgacttctttctggcccctcctatccgtacctgcagaagctaaccagattgctcttattttttttcttttttcaaaatatagcaaaatgcaggtaacacttccccagcctcagagccttctgtttgcacagtaggggcaacctcatcgaatgatgccgccacatcctggtccaactatggctcagttggtacgtagggctcggttttatttattacttcttccccacatgcgatcagaccggccgctgactatatttagttgacgtttacgctcccggagacgcaattgtctctacctggcccggtggcggttccaggtctctctcaggcacatcgatggcttctccacacgtcgccggcctgggtgcatacctcatcgctctggagggcattagcggaggcagtgtatgtgaccgtatcaaagagctggctcaacctgtcgtccagcctggtccaggcaccaccaaccgtcttatctacaacggcagtggccgctaa

SEQ ID NO: 4 - protein, 281 aa, Malbranchea cinnamomea
  M59 mature amino acid sequence
ALVTQSNAPSWGLGRISNRQAGIRDYHYDDSAGEGVIVYDVDTGIDISHPDFEGRAIWGSNHVDRVNQDQNGHGTHVAGTIGGRAYGVAKKATIVAVKVLDADGSGTISGIIAGLDWSVNHARQNGVTRRAALNMSLGGGRSISFNQAAASAVQAGLFVAVAAGNEGQNAGNTSPASEPSVCTVGATSSNDAATSWSNYGSVVDVYAPGDAIVSTWPGGGSRSLSGTSMASPHVAGLGAYLIALEGISGGSVCDRIKELAQPVVQPGPGTTNRLIYNGSGR

SEQ ID NO: 5 - DNA, 1004 bp, Malbranchea cinnamomea
  M60 mature nucleotide sequence
  misc_feature (315)..(315): y is g or a
gcattggtgacgcagagtaatgcaccatcctggggccttggccgtatttccaaccgacaggctggtattcgtgattaccactacgatgactccgccggtgaaggcgtcatcgtctatgatgttgacaccggcattgacatcagccatccggatttcgagggccgtgctatatggggttccaaccatgtcgaccgcgttaaccaggatcagaatggccatgggacacacgttgctggtactattggtggaagggcgtacggagtcgccaagaaggccacaatagtggctgtcaaggttctcgacgcccagggggayggtactatcagcggtattattgctggtcttgactggagtgtcaatcatgctcgacagaatggagtcactagaagagcggctttgaacatgagccttggcggtgggcgcagtatctctttcaatcaggctgctgcaagtgctgtccaagccggattgttcgtcgcggttgctgccggaaatgaaggggtaagtgacttctttctggcccctcctatccgtacctgcagaagctaaccagattgctcttattttttttcttttttcaaaatatagcaaaatgcaggtaacacttccccagcctcagagccttctgtttgcacagtaggggcaacctcatcgaatgatgccgccacatcctggtccaactatggctcagttggtacgtagggctcggttttatttattacttcttccccacatgcgatcagaccggccgctgactatatttagttgacgtttacgctcccggagacgcaattgtctctacctggcccggtggcggttccaggtctctctcaggcacatcgatggcttctccacacgtcgccggcctgggtgcatacctcatcgctctggagggcattagcggaggcagtgtatgtgaccgtatcaaagagctggctcaacctgtcgtccagcctggtccaggcaccaccaaccgtcttatctacaacggcagtggccgctaa

SEQ ID NO: 6 - protein, 281 aa, Malbranchea cinnamomea
  M60 mature amino acid sequence
ALVTQSNAPSWGLGRISNRQAGIRDYHYDDSAGEGVIVYDVDTGIDISHPDFEGRAIWGSNHVDRVNQDQNGHGTHVAGTIGGRAYGVAKKATIVAVKVLDAQGEGTISGIIAGLDWSVNHARQNGVTRRAALNMSLGGGRSISFNQAAASAVQAGLFVAVAAGNEGQNAGNTSPASEPSVCTVGATSSNDAATSWSNYGSVVDVYAPGDAIVSTWPGGGSRSLSGTSMASPHVAGLGAYLIALEGISGGSVCDRIKELAQPVVQPGPGTTNRLIYNGSGR

SEQ ID NO: 7 - DNA, 1004 bp, Malbranchea cinnamomea
  M61 mature nucleotide sequence
  misc_feature (309)..(309): r is t or c
  misc_feature (315)..(315): y is g or a
gcattggtgacgcagagtaatgcaccatcctggggccttggccgtatttccaaccgacaggctggtattcgtgattaccactacgatgactccgccggtgaaggcgtcatcgtctatgatgttgacaccggcattgacatcagccatccggatttcgagggccgtgctatatggggttccaaccatgtcgaccgcgttaaccaggatcagaatggccatgggacacacgttgctggtactattggtggaagggcgtacggagtcgccaagaaggccacaatagtggctgtcaaggttctcgacgccgarggggayggtactatcagcggtattattgctggtcttgactggagtgtcaatcatgctcgacagaatggagtcactagaagagcggctttgaacatgagccttggcggtgggcgcagtatctctttcaatcaggctgctgcaagtgctgtccaagccggattgttcgtcgcggttgctgccggaaatgaaggggtaagtgacttctttctggcccctcctatccgtacctgcagaagctaaccagattgctcttattttttttcttttttcaaaatatagcaaaatgcaggtaacacttccccagcctcagagccttctgtttgcacagtaggggcaacctcatcgaatgatgccgccacatcctggtccaactatggctcagttggtacgtagggctcggttttatttattacttcttccccacatgcgatcagaccggccgctgactatatttagttgacgtttacgctcccggagacgcaattgtctctacctggcccggtggcggttccaggtctctctcaggcacatcgatggcttctccacacgtcgccggcctgggtgcatacctcatcgctctggagggcattagcggaggcagtgtatgtgaccgtatcaaagagctggctcaacctgtcgtccagcctggtccaggcaccaccaaccgtcttatctacaacggcagtggccgctaa

SEQ ID NO: 8 - protein, 281 aa, Malbranchea cinnamomea
  M61 mature amino acid sequence
ALVTQSNAPSWGLGRISNRQAGIRDYHYDDSAGEGVIVYDVDTGIDISHPDFEGRAIWGSNHVDRVNQDQNGHGTHVAGTIGGRAYGVAKKATIVAVKVLDADGEGTISGIIAGLDWSVNHARQNGVTRRAALNMSLGGGRSISFNQAAASAVQAGLFVAVAAGNEGQNAGNTSPASEPSVCTVGATSSNDAATSWSNYGSVVDVYAPGDAIVSTWPGGGSRSLSGTSMASPHVAGLGAYLIALEGISGGSVCDRIKELAQPVVQPGPGTTNRLIYNGSGR

SEQ ID NO: 9 - DNA, 1436 bp, Malbranchea cinnamomea
  The nucleotide sequence encoding the full-length amino acid sequence of Malbranchea ALKO4122 protease. The full-length gene in included in plasmid pALK3094. The protease sequence cloned from Malbranchea ALKO4178 by PCR was identical to this sequence.
atgggcgtcttcagcaaactcttgtatctgtcttttgcagtcacggcctctgtcaatgccggtgaaatcctttcagtcgccaacaaggacagtgttatccctgacacgtatatcgtggtgttgaaggaaggagtttcaacccaggagttcaatgctcataaaaactgggtgaacgagattcatcgcaccaacctcacgaggcgtgacctgggtttcactggcgagttaaagcatagctatgattttggtggacatggactgaagggctacagcggcaagtttgatgccactgccattcaggaaattgccaatgatcctaatgtatgcttgttaagaattcttcccagcgagatatcttcatgcaagccatgcaattgctgacaggtgaattaggtggcctacgtcgaaccggaccaggaggtgaagcttgatgcattggtgacgcagagtaatgcaccatcctggggccttggccgtatttccaaccgacaggctggtattcgtgattaccactacgatgactccgccggtgaaggcgtcatcgtctatgatgttgacaccggtattgacatcagccatccggatttcgagggccgtgctatatggggttccaaccatgtcgaccgcgttaaccaggatcagaatggccatgggacacacgttgctggtactattggtggaagggcgtacggagtcgccaagaaggccacaatagtggctgtcaaggttctcgacgcccaggggtcaggtactatcagcggtattattgctggtcttgactggagtgtcaatcatgctcgacagaatggagtcactagaagagcggctttgaacatgagccttggcggtgggcgcagtatctctttcaatcaggctgctgcaagtgctgtccaagccggattgttcgtcgcggttgctgccggaaatgaaggggtaagtgacttctttctggcccctcctatccgtacctgcagaagctaaccagattgctcttattttttttcttttttcaaaatatagcaaaatgcaggtaacacttccccagcctcagagccttctgtttgcacagtaggggcaacctcatcgaatgatgccgccacatcctggtccaactatggctcagttggtacgtagggctcggttttatttattacttcttccccacatgcgatcagaccggccgctgactatatttagttgacgtttacgctcccggagacgcaattgtctctacctggcccggtggcggttccaggtctctctcaggcacatcgatggcttctccacacgtcgccggcctgggtgcatacctcatcgctctggagggcattagcggaggcagtgtatgtgaccgtatcaaagagctggctcaacctgtcgtccagcctggtccaggcaccaccaaccgtcttatctacaacggcagtggccgctaa

SEQ ID NO: 10 - protein, 401 aa, Malbranchea cinnamomea
  The full-length amino acid sequence of Malbranchea ALKO4122 protease including amino acids Met1 to Arg 401 of the full length protease.
MGVFSKLLYLSFAVTASVNAGEILSVANKDSVIPDTYIVVLKEGVSTQEFNAHKNWVNEIHRTNLTRRDLGFTGELKHSYDFGGHGLKGYSGKFDATAIQEIANDPNVAYVEPDQEVKLDALVTQSNAPSWGLGRISNRQAGIRDYHYDDSAGEGVIVYDVDTGIDISHPDFEGRAIWGSNHVDRVNQDQNGHGTHVAGTIGGRAYGVAKKATIVAVKVLDAQGSGTISGIIAGLDWSVNHARQNGVTRRAALNMSLGGGRSISFNQAAASAVQAGLFVAVAAGNEGQNAGNTSPASEPSVCTVGATSSNDAATSWSNYGSVVDVYAPGDAIVSTWPGGGSRSLSGTSMASPHVAGLGAYLIALEGISGGSVCDRIKELAQPVVQPGPGTTNRLIYNGSGR